European Patent Specification EP 3 436 602 B1, published August 14, 2024. Title: NANOPORE PROTEIN CONJUGATES AND USES THEREOF. Applicant: GENIA TECHNOLOGIES, INC. The sequence listing filed with the application follows.

SEQUENCE LISTING (12 sequences)

SEQ ID NO: 1 - DNA, 1023 bp, Staphylococcus aureus
atggcagatctcgatcccgcgaaattaatacgactcactatagggaggccacaacggtttccctctagaaataattttgtttaactttaagaaggagatatacaaatggattcagatattaatattaaaacaggtacaacagatattggttcaaatacaacagtaaaaactggtgatttagtaacttatgataaagaaaatggtatgcataaaaaagtattttattcttttattgatgataaaaatcataataaaaaattgttagttattcgtacaaaaggtactattgcaggtcaatatagagtatatagtgaagaaggtgctaataaaagtggtttagcatggccatctgcttttaaagttcaattacaattacctgataatgaagtagcacaaatttcagattattatccacgtaatagtattgatacaaaagaatatatgtcaacattaacttatggttttaatggtaatgtaacaggtgatgatactggtaaaattggtggtttaattggtgctaatgtttcaattggtcatacattaaaatatgtacaaccagattttaaaacaattttagaaagtcctactgataaaaaagttggttggaaagtaatttttaataatatggttaatcaaaattggggtccttatgatcgtgatagttggaatcctgtatatggtaatcaattatttatgaaaacaagaaatggttctatgaaagcagctgataatttcttagatccaaataaagcatcaagtttattatcttcaggtttttctcctgattttgcaacagttattactatggatagaaaagcatcaaaacaacaaacaaatattgatgttatttatgaacgtgtaagagatgattatcaattacattggacatcaactaattggaaaggtacaaatactaaagataaatggacagatagaagttcagaaagatataaaattgattgggaaaaagaagaaatgacaaatggtctcagcgcttggagccacccgcagttcgaaaaataa

SEQ ID NO: 2 - protein, 64 aa, Sulfolobus solfataricus
MATVKFKYKGEEKEVDISKIKKVWRVGKMISFTYDEGGGKTGRGAVSEKDAPKELLQMLEKQKK

SEQ ID NO: 3 - protein, 305 aa, Staphylococcus aureus
ADSDINIKTGTTDIGSNTTVKTGDLVTYDKENGMHKKVFYSFIDDKNHNKKLLVIRTKGTIAGQYRVYSEEGANKSGLAWPSAFKVQLQLPDNEVAQISDYYPRNSIDTKEYMSTLTYGFNGNVTGDDTGKIGGLIGANVSIGHTLKYVQPDFKTILESPTDKKVGWKVIFNNMVNQNWGPYDRDSWNPVYGNQLFMKTRNGSMKAADNFLDPNKASSLLSSGFSPDFATVITMDRKASKQQTNIDVIYERVRDDYQLHWTSTNWKGTNTKDKWTDRSSERYKIDWEKEEMTNGLSAWSHPQFEK

SEQ ID NO: 4 - protein, 293 aa, Staphylococcus aureus
ADSDINIKTGTTDIGSNTTVKTGDLVTYDKENGMHKKVFYSFIDDKNHNKKLLVIRTKGTIAGQYRVYSEEGANKSGLAWPSAFKVQLQLPDNEVAQISDYYPRNSIDTKEYMSTLTYGFNGNVTGDDTGKIGGLIGANVSIGHTLKYVQPDFKTILESPTDKKVGWKVIFNNMVNQNWGPYDRDSWNPVYGNQLFMKTRNGSMKAADNFLDPNKASSLLSSGFSPDFATVITMDRKASKQQTNIDVIYERVRDDYQLHWTSTNWKGTNTKDKWTDRSSERYKIDWEKEEMTN

SEQ ID NO: 5 - protein, 362 aa, Artificial Sequence
  alpha-HL/Sso7d conjugate
MADSDINIKTGTTDIGSNTTVKTGDLVTYDKENGMHKKVFYSFIDDKNHNKKLLVIRTKGTIAGQYRVYSEEGANKSGLAWPSAFKVQLQLPDNEVAQISDYYPRNSIDTKEYMSTLTYGFNGNVTGDDTGKIGGLIGANVSIGATLKYVQPDFKTILESPTDKKVGWKVIFNNMVNQNWGPYDRDSWNPVYGNQLFMKTRNGSMKAADNFLDPNKASSLLSSGFSPDFATVITMDRKASKQQTNIDVIYERVRDDYQLHWTSTNWKGTNTKDKWTDRSSERYKIDWEKEEMTNGLSAMATVKFKYKGEEKEVDISKIKKVWRVGKMISFTYDEGGGKTGRGAVSEKDAPKELLQMLEKQKK

SEQ ID NO: 6 - DNA, 1086 bp, Artificial Sequence
  alpha-HL/Sso7d conjugate coding sequence
atggcagattcagatattaatattaaaacaggtacaacagatattggttcaaatacaacagtaaaaactggtgatttagtaacttatgataaagaaaatggtatgcataaaaaagtattttattcttttattgatgataaaaatcataataaaaaattgttagttattcgtacaaaaggtactattgcaggtcaatatagagtatatagtgaagaaggtgctaataaaagtggtttagcatggccatctgcttttaaagttcaattacaattacctgataatgaagtagcacaaatttcagattattatccacgtaatagtattgatacaaaagaatatatgtcaacattaacttatggttttaatggtaatgtaacaggtgatgatactggtaaaattggtggtttaattggtgctaatgtttcaattggtgcgacattaaaatatgtacaaccagattttaaaacaattttagaaagtcctactgataaaaaagttggttggaaagtaatttttaataatatggttaatcaaaattggggtccttatgatcgtgatagttggaatcctgtatatggtaatcaattatttatgaaaacaagaaatggttctatgaaagcagctgataatttcttagatccaaataaagcatcaagtttattatcttcaggtttttctcctgattttgcaacagttattactatggatagaaaagcatcaaaacaacaaacaaatattgatgttatttatgaacgtgtaagagatgattatcaattacattggacatcaactaattggaaaggtacaaatactaaagataaatggacagatagaagttcagaaagatataaaattgattgggaaaaagaagaaatgacaaatggtctcagcgctatggctaccgttaaattcaaatacaaaggtgaagaaaaagaagttgacatctctaaaatcaagaaagtgtggcgtgttggtaaaatgatctctttcacctacgacgaaggtggtggtaaaaccggtcgtggtgctgtttctgaaaaagacgctccgaaagaactgctgcagatgctggaaaaacagaaaaaa

SEQ ID NO: 7 - protein, 4 aa, Artificial Sequence
  GLSA linker
GLSA

SEQ ID NO: 8 - protein, 305 aa, Artificial Sequence
  N17K alpha-HL
ADSDINIKTGTTDIGSKTTVKTGDLVTYDKENGMHKKVFYSFIDDKNHNKKLLVIRTKGTIAGQYRVYSEEGANKSGLAWPSAFKVQLQLPDNEVAQISDYYPRNSIDTKEYMSTLTYGFNGNVTGDDTGKIGGLIGANVSIGHTLKYVQPDFKTILESPTDKKVGWKVIFNNMVNQNWGPYDRDSWNPVYGNQLFMKTRNGSMKAADNFLDPNKASSLLSSGFSPDFATVITMDRKASKQQTNIDVIYERVRDDYQLHWTSTNWKGTNTKDKWTDRSSERYKIDWEKEEMTNGLSAWSHPQFEK

SEQ ID NO: 9 - protein, 305 aa, Artificial Sequence
  N17R alpha-HL
ADSDINIKTGTTDIGSRTTVKTGDLVTYDKENGMHKKVFYSFIDDKNHNKKLLVIRTKGTIAGQYRVYSEEGANKSGLAWPSAFKVQLQLPDNEVAQISDYYPRNSIDTKEYMSTLTYGFNGNVTGDDTGKIGGLIGANVSIGHTLKYVQPDFKTILESPTDKKVGWKVIFNNMVNQNWGPYDRDSWNPVYGNQLFMKTRNGSMKAADNFLDPNKASSLLSSGFSPDFATVITMDRKASKQQTNIDVIYERVRDDYQLHWTSTNWKGTNTKDKWTDRSSERYKIDWEKEEMTNGLSAWSHPQFEK

SEQ ID NO: 10 - protein, 305 aa, Artificial Sequence
  T12K alpha-HL
ADSDINIKTGTKDIGSNTTVKTGDLVTYDKENGMHKKVFYSFIDDKNHNKKLLVIRTKGTIAGQYRVYSEEGANKSGLAWPSAFKVQLQLPDNEVAQISDYYPRNSIDTKEYMSTLTYGFNGNVTGDDTGKIGGLIGANVSIGHTLKYVQPDFKTILESPTDKKVGWKVIFNNMVNQNWGPYDRDSWNPVYGNQLFMKTRNGSMKAADNFLDPNKASSLLSSGFSPDFATVITMDRKASKQQTNIDVIYERVRDDYQLHWTSTNWKGTNTKDKWTDRSSERYKIDWEKEEMTNGLSAWSHPQFEK

SEQ ID NO: 11 - protein, 305 aa, Artificial Sequence
  T12R alpha-HL
ADSDINIKTGTRDIGSNTTVKTGDLVTYDKENGMHKKVFYSFIDDKNHNKKLLVIRTKGTIAGQYRVYSEEGANKSGLAWPSAFKVQLQLPDNEVAQISDYYPRNSIDTKEYMSTLTYGFNGNVTGDDTGKIGGLIGANVSIGHTLKYVQPDFKTILESPTDKKVGWKVIFNNMVNQNWGPYDRDSWNPVYGNQLFMKTRNGSMKAADNFLDPNKASSLLSSGFSPDFATVITMDRKASKQQTNIDVIYERVRDDYQLHWTSTNWKGTNTKDKWTDRSSERYKIDWEKEEMTNGLSAWSHPQFEK

SEQ ID NO: 12 - DNA, 1125 bp, Artificial Sequence
  alpha-HL/Sso7d coding sequence with His-Tag
atggcagattcagatattaatattaaaacaggtacaacagatattggttcaaatacaacagtaaaaactggtgatttagtaacttatgataaagaaaatggtatgcataaaaaagtattttattcttttattgatgataaaaatcataataaaaaattgttagttattcgtacaaaaggtactattgcaggtcaatatagagtatatagtgaagaaggtgctaataaaagtggtttagcatggccatctgcttttaaagttcaattacaattacctgataatgaagtagcacaaatttcagattattatccacgtaatagtattgatacaaaagaatatatgtcaacattaacttatggttttaatggtaatgtaacaggtgatgatactggtaaaattggtggtttaattggtgctaatgtttcaattggtgcgacattaaaatatgtacaaccagattttaaaacaattttagaaagtcctactgataaaaaagttggttggaaagtaatttttaataatatggttaatcaaaattggggtccttatgatcgtgatagttggaatcctgtatatggtaatcaattatttatgaaaacaagaaatggttctatgaaagcagctgataatttcttagatccaaataaagcatcaagtttattatcttcaggtttttctcctgattttgcaacagttattactatggatagaaaagcatcaaaacaacaaacaaatattgatgttatttatgaacgtgtaagagatgattatcaattacattggacatcaactaattggaaaggtacaaatactaaagataaatggacagatagaagttcagaaagatataaaattgattgggaaaaagaagaaatgacaaatggtctcagcgctatggctaccgttaaattcaaatacaaaggtgaagaaaaagaagttgacatctctaaaatcaagaaagtgtggcgtgttggtaaaatgatctctttcacctacgacgaaggtggtggtaaaaccggtcgtggtgctgtttctgaaaaagacgctccgaaagaactgctgcagatgctggaaaaacagaaaaaagaaaacctgtatttccagggtcatcaccatcaccatcac